European Patent Application EP 4 279 601 A1, published November 22, 2023. Title: PROTEIN HAVING L-PROLINE EFFLUX FUNCTION, AND USE THEREOF. Applicant: Tianjin Institute of Industrial Biotechnology, Chinese Academy of Sciences. The sequence listing filed with the application follows.

SEQUENCE LISTING (23 sequences)

SEQ ID NO: 1 - protein, 489 aa, Corynebacterium glutamicum
MLSFATLRGRISTVDAAKAAPPPSPLAPIDLTDHSQVAGVMNLAARIGDILLSSGTSNSDTKVQVRAVTSAYGLYYTHVDITLNTITIFTNIGVERKMPVNVFHVVGKLDTNFSKLSEVDRLIRSIQAGATPPEVAEKILDELEQSPASYGFPVALLGWAMMGGAIAVLLGGGWQVSLIAFITAFTIISTTSFLGKKGLPTFFQNVVGGFIATLPASIAYSLALHFGLEIKPSQIIASGIVVLLAGLTLVQSLQDGITGAPVTASARFFETLLFTGGIVAGVGLGIQLSEILHVMLPAMESAAAPNYSSTFARIIAGGVTAAAFAVGCYAEWSSVIIAGLTALMGSAFYYLFVVYLGPVSAAAIAATAVGFTGGLLARRFLIPPLIVAIAGITPMLPGLAIYRGMYATLNDQTLMGFTNIAVALATASSLAAGVVLGEWIARRLRRPPRFNPYRAFTKANEFSFQEEAEQNQRRQRKRPKTNQRFGNKR

SEQ ID NO: 2 - protein, 489 aa, Corynebacterium glutamicum
MLSFATLRGRISTVDAAKAAPPPSPLAPIDLTDHSQVAGVMNLAARIGDILLSSGTSNSDTKVQVRAVTSAYGLYYTHVDITLNTITIFTNIGVERKMPVNVFHVVGKLDTNFSKLSEVDRLIRSIQAGATPPEVAEKILDELEQSPASYGFPVALLGWAMMGGAVAVLLGGGWQVSLIAFITAFTIIATTSFLGKKGLPTFFQNVVGGFIATLPASIAYSLALQFGLEIKPSQIIASGIVVLLAGLTLVQSLQDGITGAPVTASARFFETLLFTGGIVAGVGLGIQLSEILHVMLPAMESAAAPNYSSTFARIIAGGVTAAAFAVGCYAEWSSVIIAGLTALMGSAFYYLFVVYLGPVSAAAIAATAVGFTGGLLARRFLIPPLIVAIAGITPMLPGLAIYRGMYATLNDQTLMGFTNIAVALATASSLAAGVVLGEWIARRLRRPPRFNPYRAFTKANEFSFQEEAEQNQRRQRKRPKTNQRFGNKR

SEQ ID NO: 3 - DNA, 11773 bp, Artificial Sequence
aattaagcttaaaggagttgagaatggataagaaatactcaataggcttagctatcggcacaaatagcgtcggatgggcggtgatcactgatgaatataaggttccgtctaaaaagttcaaggttctgggaaatacagaccgccacagtatcaaaaaaaatcttataggggctcttttatttgacagtggagagacagcggaagcgactcgtctcaaacggacagctcgtagaaggtatacacgtcggaagaatcgtatttgttatctacaggagattttttcaaatgagatggcgaaagtagatgatagtttctttcatcgacttgaagagtcttttttggtggaagaagacaagaagcatgaacgtcatcctatttttggaaatatagtagatgaagttgcttatcatgagaaatatccaactatctatcatctgcgaaaaaaattggtagattctactgataaagcggatttgcgcttaatctatttggccttagcgcatatgattaagtttcgtggtcattttttgattgagggagatttaaatcctgataatagtgatgtggacaaactatttatccagttggtacaaacctacaatcaattatttgaagaaaaccctattaacgcaagtggagtagatgctaaagcgattctttctgcacgattgagtaaatcaagacgattagaaaatctcattgctcagctccccggtgagaagaaaaatggcttatttgggaatctcattgctttgtcattgggtttgacccctaattttaaatcaaattttgatttggcagaagatgctaaattacagctttcaaaagatacttacgatgatgatttagataatttattggcgcaaattggagatcaatatgctgatttgtttttggcagctaagaatttatcagatgctattttactttcagatatcctaagagtaaatactgaaataactaaggctcccctatcagcttcaatgattaaacgctacgatgaacatcatcaagacttgactcttttaaaagctttagttcgacaacaacttccagaaaagtataaagaaatcttttttgatcaatcaaaaaacggatatgcaggttatattgatgggggagctagccaagaagaattttataaatttatcaaaccaattttagaaaaaatggatggtactgaggaattattggtgaaactaaatcgtgaagatttgctgcgcaagcaacggacctttgacaacggctctattccccatcaaattcacttgggtgagctgcatgctattttgagaagacaagaagacttttatccatttttaaaagacaatcgtgagaagattgaaaaaatcttgacttttcgaattccttattatgttggtccattggcgcgtggcaatagtcgttttgcatggatgactcggaagtctgaagaaacaattaccccatggaattttgaagaagttgtcgataaaggtgcttcagctcaatcatttattgaacgcatgacaaactttgataaaaatcttccaaatgaaaaagtactaccaaaacatagtttgctttatgagtattttacggtttataacgaattgacaaaggtcaaatatgttactgaaggaatgcgaaaaccagcatttctttcaggtgaacagaagaaagccattgttgatttactcttcaaaacaaatcgaaaagtaaccgttaagcaattaaaagaagattatttcaaaaaaatagaatgttttgatagtgttgaaatttcaggagttgaagatagatttaatgcttcattaggtacctaccatgatttgctaaaaattattaaagataaagattttttggataatgaagaaaatgaagatatcttagaggatattgttttaacattgaccttatttgaagatagggagatgattgaggaaagacttaaaacatatgctcacctctttgatgataaggtgatgaaacagcttaaacgtcgccgttatactggttggggacgtttgtctcgaaaattgattaatggtattagggataagcaatctggcaaaacaatattagattttttgaaatcagatggttttgccaatcgcaattttatgcagctgatccatgatgatagtttgacatttaaagaagacattcaaaaagcacaagtgtctggacaaggcgatagtttacatgaacatattgcaaatttagctggtagccctgctattaaaaaaggtattttacagactgtaaaagttgttgatgaattggtcaaagtaatggggcggcataagccagaaaatatcgttattgaaatggcacgtgaaaatcagacaactcaaaagggccagaaaaattcgcgagagcgtatgaaacgaatcgaagaaggtatcaaagaattaggaagtcagattcttaaagagcatcctgttgaaaatactcaattgcaaaatgaaaagctctatctctattatctccaaaatggaagagacatgtatgtggaccaagaattagatattaatcgtttaagtgattatgatgtcgatgccattgttccacaaagtttccttaaagacgattcaatagacaataaggtcttaacgcgttctgataaaaatcgtggtaaatcggataacgttccaagtgaagaagtagtcaaaaagatgaaaaactattggagacaacttctaaacgccaagttaatcactcaacgtaagtttgataatttaacgaaagctgaacgtggaggtttgagtgaacttgataaagctggttttatcaaacgccaattggttgaaactcgccaaatcactaagcatgtggcacaaattttggatagtcgcatgaatactaaatacgatgaaaatgataaacttattcgagaggttaaagtgattaccttaaaatctaaattagtttctgacttccgaaaagatttccaattctataaagtacgtgagattaacaattaccatcatgcccatgatgcgtatctaaatgccgtcgttggaactgctttgattaagaaatatccaaaacttgaatcggagtttgtctatggtgattataaagtttatgatgttcgtaaaatgattgctaagtctgagcaagaaataggcaaagcaaccgcaaaatatttcttttactctaatatcatgaacttcttcaaaacagaaattacacttgcaaatggagagattcgcaaacgccctctaatcgaaactaatggggaaactggagaaattgtctgggataaagggcgagattttgccacagtgcgcaaagtattgtccatgccccaagtcaatattgtcaagaaaacagaagtacagacaggcggattctccaaggagtcaattttaccaaaaagaaattcggacaagcttattgctcgtaaaaaagactgggatccaaaaaaatatggtggttttgatagtccaacggtagcttattcagtcctagtggttgctaaggtggaaaaagggaaatcgaagaagttaaaatccgttaaagagttactagggatcacaattatggaaagaagttcctttgaaaaaaatccgattgactttttagaagctaaaggatataaggaagttaaaaaagacttaatcattaaactacctaaatatagtctttttgagttagaaaacggtcgtaaacggatgctggctagtgccggagaattacaaaaaggaaatgagctggctctgccaagcaaatatgtgaattttttatatttagctagtcattatgaaaagttgaagggtagtccagaagataacgaacaaaaacaattgtttgtggagcagcataagcattatttagatgagattattgagcaaatcagtgaattttctaagcgtgttattttagcagatgccaatttagataaagttcttagtgcatataacaaacatagagacaaaccaatacgtgaacaagcagaaaatattattcatttatttacgttgacgaatcttggagctcccgctgcttttaaatattttgatacaacaattgatcgtaaacgatatacgtctacaaaagaagttttagatgccactcttatccatcaatccatcactggtctttatgaaacacgcattgatttgagtcagctaggaggtgactgagcttggctgttttggcggatgagagaagattttcagcctgatacagattaaatcagaacgcagaagcggtctgataaaacagaatttgcctggcggcagtagcgcggtggtcccacctgaccccatgccgaactcagaagtgaaacgccgtagcgccgatggtagtgtggggtctgcccatgcgagagtagggaactgccaggcatcaaataaaacgaaaggctcagtcgaaagactgggcctttcgttttatctgttgtttgtcggtgaacgctctcctgagtaggacaaatccgccgggagcggatttgaacgttgcgaagcaacggcccggagggtggcgggcaggacgcccgccataaactgccaggcatcaaattaagcagaaggccatcctgacggatggcctttttgcgtttctacaaactcttttgtttatttttctaaatacattcaaatatgtatccgctcatgagacaataaccctgataaatgcttcaataatattgaaaaaggaagagtatgagtattcaacatttccgtgtcgcccttattcccttttttgcggcattttgccttcctgtttttgctcacccagaaacgctggtgaaagtaaaagatgctgaagatcagttgggtgcacgagtgggttacatcgaactggatctcaacagcggtaagatccttgagagttttcgccccgaagaacgttttccaatgatgagcacttttgcttcctcgctcactgactcgctgcgctcggtcgttcggctgcggcgagcggtatcagctcactcaaaggcggtaatacggttatccacagaatcaggggataacgcaggaaagaacatgtgagcaaaaggccagcaaaaggccaggaaccgtaaaaaggccgcgttgctggcgtttttccataggctccgcccccctgacgagcatcacaaaaatcgacgctcaagtcagaggtggcgaaacccgacaggactataaagataccaggcgtttccccctggaagctccctcgtgcgctctcctgttccgaccctgccgcttaccggatacctgtccgcctttctcccttcgggaagcgtggcgctttctcaatgctcacgctgtaggtatctcagttcggtgtaggtcgttcgctccaagctgggctgtgtgcacgaaccccccgttcagcccgaccgctgcgccttatccggtaactatcgtcttgagtccaacccggtaagacacgacttatcgccactggcagcagccactggtaacaggattagcagagcgaggtatgtaggcggtgctacagagttcttgaagtggtggcctaactacggctacactagaaggacagtatttggtatctgcgctctgctgaagccagttaccttcggaaaaagagttggtagctcttgatccggcaaacaaaccaccgctggtagcggtggtttttttgtttgcaagcagcagattacgcgcagaaaaaaaggatctcaagaagatcctttgatcttttctacggggtctgacgctcagtggaacgaaaactcacgttaagggattttggtcatgagattatcaaaaaggatcttcacctagatccttttggggtgggcgaagaactccagcatgagatccccgcgctggaggatcatccagccattcggggtcgttcactggttcccctttctgatttctggcatagaagaacccccgtgaactgtgtggttccgggggttgctgatttttgcgagacttctcgcgcaattccctagcttaggtgaaaacaccatgaaacactagggaaacacccatgaaacacccattagggcagtagggcggcttcttcgtctagggcttgcatttgggcggtgatctggtctttagcgtgtgaaagtgtgtcgtaggtggcgtgctcaatgcactcgaacgtcacgtcatttaccgggtcacggtgggcaaagagaactagtgggttagacattgttttcctcgttgtcggtggtggtgagcttttctagccgctcggtaaacgcggcgatcatgaactcttggaggttttcaccgttctgcatgcctgcgcgcttcatgtcctcacgtagtgccaaaggaacgcgtgcggtgaccacgacgggcttagcctttgcctgcgcttctagtgcttcgatggtggcttgtgcctgcgcttgctgcgcctgtagtgcctgttgagcttcttgtagttgctgttctagctgtgccttggttgccatgctttaagactctagtagctttcctgcgatatgtcatgcgcatgcgtagcaaacattgtcctgcaactcattcattatgtgcagtgctcctgttactagtcgtacatactcatatttacctagtctgcatgcagtgcatgcacatgcagtcatgtcgtgctaatgtgtaaaacatgtacatgcagattgctgggggtgcagggggcggagccaccctgtccatgcggggtgtggggcttgccccgccggtacagacagtgagcaccggggcacctagtcgcggataccccccctaggtatcggacacgtaaccctcccatgtcgatgcaaatctttaacattgagtacgggtaagctggcacgcatagccaagctaggcggccaccaaacaccactaaaaattaatagtccctagacaagacaaacccccgtgcgagctaccaactcatatgcacgggggccacataacccgaaggggtttcaattgacaaccatagcactagctaagacaacgggcacaacacccgcacaaactcgcactgcgcaaccccgcacaacatcgggtctaggtaacactgagtaacactgaaatagaagtgaacacctctaaggaaccgcaggtcaatgagggttctaaggtcactcgcgctagggcgtggcgtaggcaaaacgtcatgtacaagatcaccaatagtaaggctctggcggggtgccataggtggcgcagggacgaagctgttgcggtgtcctggtcgtctaacggtgcttcgcagtttgagggtctgcaaaactctcactctcgctgggggtcacctctggctgaattggaagtcatgggcgaacgccgcattgagctggctattgctactaagaatcacttggcggcgggtggcgcgctcatgatgtttgtgggcactgttcgacacaaccgctcacagtcatttgcgcaggttgaagcgggtattaagactgcgtactcttcgatggtgaaaacatctcagtggaagaaagaacgtgcacggtacggggtggagcacacctatagtgactatgaggtcacagactcttgggcgaacggttggcacttgcaccgcaacatgctgttgttcttggatcgtccactgtctgacgatgaactcaaggcgtttgaggattccatgttttcccgctggtctgctggtgtggttaaggccggtatggacgcgccactgcgtgagcacggggtcaaacttgatcaggtgtctacctggggtggagacgctgcgaaaatggcaacctacctcgctaagggcatgtctcaggaactgactggctccgctactaaaaccgcgtctaaggggtcgtacacgccgtttcagatgttggatatgttggccgatcaaagcgacgccggcgaggatatggacgctgttttggtggctcggtggcgtgagtatgaggttggttctaaaaacctgcgttcgtcctggtcacgtggggctaagcgtgctttgggcattgattacatagacgctgatgtacgtcgtgaaatggaagaagaactgtacaagctcgccggtctggaagcaccggaacgggtcgaatcaacccgcgttgctgttgctttggtgaagcccgatgattggaaactgattcagtctgatttcgcggttaggcagtacgttctcgattgcgtggataaggctaaggacgtggccgctgcgcaacgtgtcgctaatgaggtgctggcaagtctgggtgtggattccaccccgtgcatgatcgttatggatgatgtggacttggacgcggttctgcctactcatggggacgctactaagcgtgatctgaatgcggcggtgttcgcgggtaatgagcagactattcttcgcacccactaaaagcggcataaaccccgttcgatattttgtgcgatgaatttatggtcaatgtcgcgggggcaaactatgatgggtcttgttgttggcgtcccggaaaacgattccgaagcccaacctttcatagaaggcggcggtggaatttttctccacataagctggcaatgttgcgacgcaacaggtacagtgtaattcatgagaccacgcgtggatccggcttactaaaagccagataacagtatgcgtatttgcgcgctgatttttgcggtataagaatatatactgatatgtatacccgaagtatgtcaaaaagaggtatgctatgaagcagcgtattacagtgacagttgacagcgacagctatcagttgctcaaggcatatatgatgtcaatatctccggtctggtaagcacaaccatgcagaatgaagcccgtcgtctgcgtgccgaacgctggaaagcggaaaatcaggaagggatggctgaggtcgcccggtttattgaaatgaacggctcttttgctgacgagaacaggggctggtgaaatgcagtttaaggtttacacctataaaagagagagccgttatcgtctgtttgtggatgtacagagtgatattattgacacgcccgggcgacggatggtgatccccctggccagtgcacgtctgctgtcagataaagtctcccgtgaactttacccggtggtgcatatcggggatgaaagctggcgcatgatgaccaccgatatggccagtgtgccggtatccgttatcggggaagaagtggctgatctcagccaccgcgaaaatgacatcaaaaacgccattaacctgatgttctggggaatataaggtctcagttttagagctagaaatagcaagttaaaataaggctagtccgttatcaacttgaaaaagtggcaccgagtcggtgctttttttccaggcatcaaataaaacgaaaggctcagtcgaaagactgggcctttcgttttatctgttgtttgtcggtgaacgctctcctgagtaggacaaatccgccgggagcggatttgaacgttgcgaagcaacggcccggagggtggcgggcaggacgcccgccataaactgccaggcatcaaattaagcagaaggccatcctgacggatggcctttttgcgtttctacaaactctttttgtttatttttctaaatacattcaaatatgtatccgctcatgaattaattccgctagatgacgtgcggcttcgaaaatctcgtgatggcaggttgggcgtcgcttggtcggtcatttcgaagggcaccaataactgccttaaaaaaattacgccccgccctgccactcatcgcagtactgttgtaattcattaagcattctgccgacatggaagccatcacagacggcatgatgaacctgaatcgccagcggcatcagcaccttgtcgccttgcgtataatatttgcccatggtgaaaacgggggcgaagaagttgtccatattggccacgtttaaatcaaaactggtgaaactcacccagggattggctgagacgaaaaacatattctcaataaaccctttagggaaataggccaggttttcaccgtaacacgccacatcttgcgaatatatgtgtagaaactgccggaaatcgtcgtggtattcactccagagcgatgaaaacgtttcagtttgctcatggaaaacggtgtaacaagggtgaacactatcccatatcaccagctcaccgtctttcattgccatacggaactccggatgagcattcatcaggcgggcaagaatgtgaataaaggccggataaaacttgtgcttatttttctttacggtctttaaaaaggccgtaatatccagctgaacggtctggttataggtacattgagcaactgactgaaatgcctcaaaatgttctttacgatgccattgggatatatcaacggtggtatatccagtgatttttttctccattttagcttccttagctcctgaaaatctcgtcgaagctcggcggatttgtcctactcaagctgatccgacaaaatccacacattatcccaggtgtccggatcggtcaaatacgctgccagctcatagaccgtatccaaagcatccggggctgatccccggcgccagggtggtttttcttttcaccagtgagacgggcaacagctgattgcccttcaccgcctggccctgagagagttgcagcaagcggtccacgtggtttgccccagcaggcgaaaatcctgtttgatggtggttaacggcgggatataacatgagctgtcttcggtatcgtcgtatcccactaccgagatatccgcaccaacgcgcagcccggactcggtaatggcgcgcattgcgcccagcgccatctgatcgttggcaaccagcatcgcagtgggaacgatgccctcattcagcatttgcatggtttgttgaaaaccggacatggcactccagtcgccttcccgttccgctatcggctgaatttgattgcgagtgagatatttatgccagccagccagacgcagacgcgccgagacagaacttaatgggcccgctaacagcgcgatttgctggtgacccaatgcgaccagatgctccacgcccagtcgcgtaccgtcttcatgggagaaaataatactgttgatgggtgtctggtcagagacatcaagaaataacgccggaacattagtgcaggcagcttccacagcaatggcatcctggtcatccagcggatagttaatgatcagcccactgacgcgttgcgcgagaagattgtgcaccgccgctttacaggcttcgacgccgcttcgttctaccatcgacaccaccacgctggcacccagttgatcggcgcgagatttaatcgccgcgacaatttgcgacggcgcgtgcagggccagactggaggtggcaacgccaatcagcaacgactgtttgcccgccagttgttgtgccacgcggttgggaatgtaattcagctccgccatcgccgcttccactttttcccgcgttttcgcagaaacgtggctggcctggttcaccacgcgggaaacggtctgataagagacaccggcatactctgcgacatcgtataacgttactggtttcacattcaccaccctgaattgactctcttccgggcgctatcatgccataccgcgaaaggttttgcaccattcgatggtgtcaacgtaaatgccgcttcgccttcgcgcgcgaattgcaagctgatccgggcttatcgactgcacggtgcaccaatgcttctggcgtcaggcagccatcggaagctgtggtatggctgtgcaggtcgtaaatcactgcataattcgtgtcgctcaaggcgcactcccgttctggataatgttttttgcgccgacatcataacggttctggcaaatattctgaaatgagctgttgacaattaatcatcggctcgtataatgtgtggaattgtgagcggataacaatttcacacaggaaacagaatt

SEQ ID NO: 4 - DNA, 11773 bp, Artificial Sequence
aattaagcttaaaggcacccgatatggataagaaatactcaataggcttagatatcggcacaaatagcgtcggatgggcggtgatcactgatgaatataaggttccgtctaaaaagttcaaggttctgggaaatacagaccgccacagtatcaaaaaaaatcttataggggctcttttatttgacagtggagagacagcggaagcgactcgtctcaaacggacagctcgtagaaggtatacacgtcggaagaatcgtatttgttatctacaggagattttttcaaatgagatggcgaaagtagatgatagtttctttcatcgacttgaagagtcttttttggtggaagaagacaagaagcatgaacgtcatcctatttttggaaatatagtagatgaagttgcttatcatgagaaatatccaactatctatcatctgcgaaaaaaattggtagattctactgataaagcggatttgcgcttaatctatttggccttagcgcatatgattaagtttcgtggtcattttttgattgagggagatttaaatcctgataatagtgatgtggacaaactatttatccagttggtacaaacctacaatcaattatttgaagaaaaccctattaacgcaagtggagtagatgctaaagcgattctttctgcacgattgagtaaatcaagacgattagaaaatctcattgctcagctccccggtgagaagaaaaatggcttatttgggaatctcattgctttgtcattgggtttgacccctaattttaaatcaaattttgatttggcagaagatgctaaattacagctttcaaaagatacttacgatgatgatttagataatttattggcgcaaattggagatcaatatgctgatttgtttttggcagctaagaatttatcagatgctattttactttcagatatcctaagagtaaatactgaaataactaaggctcccctatcagcttcaatgattaaacgctacgatgaacatcatcaagacttgactcttttaaaagctttagttcgacaacaacttccagaaaagtataaagaaatcttttttgatcaatcaaaaaacggatatgcaggttatattgatgggggagctagccaagaagaattttataaatttatcaaaccaattttagaaaaaatggatggtactgaggaattattggtgaaactaaatcgtgaagatttgctgcgcaagcaacggacctttgacaacggctctattccccatcaaattcacttgggtgagctgcatgctattttgagaagacaagaagacttttatccatttttaaaagacaatcgtgagaagattgaaaaaatcttgacttttcgaattccttattatgttggtccattggcgcgtggcaatagtcgttttgcatggatgactcggaagtctgaagaaacaattaccccatggaattttgaagaagttgtcgataaaggtgcttcagctcaatcatttattgaacgcatgacaaactttgataaaaatcttccaaatgaaaaagtactaccaaaacatagtttgctttatgagtattttacggtttataacgaattgacaaaggtcaaatatgttactgaaggaatgcgaaaaccagcatttctttcaggtgaacagaagaaagccattgttgatttactcttcaaaacaaatcgaaaagtaaccgttaagcaattaaaagaagattatttcaaaaaaatagaatgttttgatagtgttgaaatttcaggagttgaagatagatttaatgcttcattaggtacctaccatgatttgctaaaaattattaaagataaagattttttggataatgaagaaaatgaagatatcttagaggatattgttttaacattgaccttatttgaagatagggagatgattgaggaaagacttaaaacatatgctcacctctttgatgataaggtgatgaaacagcttaaacgtcgccgttatactggttggggacgtttgtctcgaaaattgattaatggtattagggataagcaatctggcaaaacaatattagattttttgaaatcagatggttttgccaatcgcaattttatgcagctgatccatgatgatagtttgacatttaaagaagacattcaaaaagcacaagtgtctggacaaggcgatagtttacatgaacatattgcaaatttagctggtagccctgctattaaaaaaggtattttacagactgtaaaagttgttgatgaattggtcaaagtaatggggcggcataagccagaaaatatcgttattgaaatggcacgtgaaaatcagacaactcaaaagggccagaaaaattcgcgagagcgtatgaaacgaatcgaagaaggtatcaaagaattaggaagtcagattcttaaagagcatcctgttgaaaatactcaattgcaaaatgaaaagctctatctctattatctccaaaatggaagagacatgtatgtggaccaagaattagatattaatcgtttaagtgattatgatgtcgatcacattgttccacaaagtttccttaaagacgattcaatagacaataaggtcttaacgcgttctgataaaaatcgtggtaaatcggataacgttccaagtgaagaagtagtcaaaaagatgaaaaactattggagacaacttctaaacgccaagttaatcactcaacgtaagtttgataatttaacgaaagctgaacgtggaggtttgagtgaacttgataaagctggttttatcaaacgccaattggttgaaactcgccaaatcactaagcatgtggcacaaattttggatagtcgcatgaatactaaatacgatgaaaatgataaacttattcgagaggttaaagtgattaccttaaaatctaaattagtttctgacttccgaaaagatttccaattctataaagtacgtgagattaacaattaccatcatgcccatgatgcgtatctaaatgccgtcgttggaactgctttgattaagaaatatccaaaacttgaatcggagtttgtctatggtgattataaagtttatgatgttcgtaaaatgattgctaagtctgagcaagaaataggcaaagcaaccgcaaaatatttcttttactctaatatcatgaacttcttcaaaacagaaattacacttgcaaatggagagattcgcaaacgccctctaatcgaaactaatggggaaactggagaaattgtctgggataaagggcgagattttgccacagtgcgcaaagtattgtccatgccccaagtcaatattgtcaagaaaacagaagtacagacaggcggattctccaaggagtcaattttaccaaaaagaaattcggacaagcttattgctcgtaaaaaagactgggatccaaaaaaatatggtggttttgatagtccaacggtagcttattcagtcctagtggttgctaaggtggaaaaagggaaatcgaagaagttaaaatccgttaaagagttactagggatcacaattatggaaagaagttcctttgaaaaaaatccgattgactttttagaagctaaaggatataaggaagttaaaaaagacttaatcattaaactacctaaatatagtctttttgagttagaaaacggtcgtaaacggatgctggctagtgccggagaattacaaaaaggaaatgagctggctctgccaagcaaatatgtgaattttttatatttagctagtcattatgaaaagttgaagggtagtccagaagataacgaacaaaaacaattgtttgtggagcagcataagcattatttagatgagattattgagcaaatcagtgaattttctaagcgtgttattttagcagatgccaatttagataaagttcttagtgcatataacaaacatagagacaaaccaatacgtgaacaagcagaaaatattattcatttatttacgttgacgaatcttggagctcccgctgcttttaaatattttgatacaacaattgatcgtaaacgatatacgtctacaaaagaagttttagatgccactcttatccatcaatccatcactggtctttatgaaacacgcattgatttgagtcagctaggaggtgactgaagcttggctgttttggcggatgagagaagattttcagcctgatacagattaaatcagaacgcagaagcggtctgataaaacagaatttgcctggcggcagtagcgcggtggtcccacctgaccccatgccgaactcagaagtgaaacgccgtagcgccgatggtagtgtggggtctgcccatgcgagagtagggaactgccaggcatcaaataaaacgaaaggctcagtcgaaagactgggcctttcgttttatctgttgtttgtcggtgaacgctctcctgagtaggacaaatccgccgggagcggatttgaacgttgcgaagcaacggcccggagggtggcgggcaggacgcccgccataaactgccaggcatcaaattaagcagaaggccatcctgacggatggcctttttgcgtttctacaaactcttttgtttatttttctaaatacattcaaatatgtatccgctcatgagacaataaccctgataaatgcttcaataatattgaaaaaggaagagtatgagtattcaacatttccgtgtcgcccttattcccttttttgcggcattttgccttcctgtttttgctcacccagaaacgctggtgaaagtaaaagatgctgaagatcagttgggtgcacgagtgggttacatcgaactggatctcaacagcggtaagatccttgagagttttcgccccgaagaacgttttccaatgatgagcacttttgcttcctcgctcactgactcgctgcgctcggtcgttcggctgcggcgagcggtatcagctcactcaaaggcggtaatacggttatccacagaatcaggggataacgcaggaaagaacatgtgagcaaaaggccagcaaaaggccaggaaccgtaaaaaggccgcgttgctggcgtttttccataggctccgcccccctgacgagcatcacaaaaatcgacgctcaagtcagaggtggcgaaacccgacaggactataaagataccaggcgtttccccctggaagctccctcgtgcgctctcctgttccgaccctgccgcttaccggatacctgtccgcctttctcccttcgggaagcgtggcgctttctcaatgctcacgctgtaggtatctcagttcggtgtaggtcgttcgctccaagctgggctgtgtgcacgaaccccccgttcagcccgaccgctgcgccttatccggtaactatcgtcttgagtccaacccggtaagacacgacttatcgccactggcagcagccactggtaacaggattagcagagcgaggtatgtaggcggtgctacagagttcttgaagtggtggcctaactacggctacactagaaggacagtatttggtatctgcgctctgctgaagccagttaccttcggaaaaagagttggtagctcttgatccggcaaacaaaccaccgctggtagcggtggtttttttgtttgcaagcagcagattacgcgcagaaaaaaaggatctcaagaagatcctttgatcttttctacggggtctgacgctcagtggaacgaaaactcacgttaagggattttggtcatgagattatcaaaaaggatcttcacctagatccttttggggtgggcgaagaactccagcatgagatccccgcgctggaggatcatccagccattcggggtcgttcactggttcccctttctgatttctggcatagaagaacccccgtgaactgtgtggttccgggggttgctgatttttgcgagacttctcgcgcaattccctagcttaggtgaaaacaccatgaaacactagggaaacacccatgaaacacccattagggcagtagggcggcttcttcgtctagggcttgcatttgggcggtgatctggtctttagcgtgtgaaagtgtgtcgtaggtggcgtgctcaatgcactcgaacgtcacgtcatttaccgggtcacggtgggcaaagagaactagtgggttagacattgttttcctcgttgtcggtggtggtgagcttttctagccgctcggtaaacgcggcgatcatgaactcttggaggttttcaccgttctgcatgcctgcgcgcttcatgtcctcacgtagtgccaaaggaacgcgtgcggtgaccacgacgggcttagcctttgcctgcgcttctagtgcttcgatggtggcttgtgcctgcgcttgctgcgcctgtagtgcctgttgagcttcttgtagttgctgttctagctgtgccttggttgccatgctttaagactctagtagctttcctgcgatatgtcatgcgcatgcgtagcaaacattgtcctgcaactcattcattatgtgcagtgctcctgttactagtcgtacatactcatatttacctagtctgcatgcagtgcatgcacatgcagtcatgtcgtgctaatgtgtaaaacatgtacatgcagattgctgggggtgcagggggcggagccaccctgtccatgcggggtgtggggcttgccccgccggtacagacagtgagcaccggggcacctagtcgcggataccccccctaggtatcggacacgtaaccctcccatgtcgatgcaaatctttaacattgagtacgggtaagctggcacgcatagccaagctaggcggccaccaaacaccactaaaaattaatagtccctagacaagacaaacccccgtgcgagctaccaactcatatgcacgggggccacataacccgaaggggtttcaattgacaaccatagcactagctaagacaacgggcacaacacccgcacaaactcgcactgcgcaaccccgcacaacatcgggtctaggtaacactgagtaacactgaaatagaagtgaacacctctaaggaaccgcaggtcaatgagggttctaaggtcactcgcgctagggcgtggcgtaggcaaaacgtcatgtacaagatcaccaatagtaaggctctggcggggtgccataggtggcgcagggacgaagctgttgcggtgtcctggtcgtctaacggtgcttcgcagtttgagggtctgcaaaactctcactctcgctgggggtcatctctggctgaattggaagtcatgggcgaacgccgcattgagctggctattgctactaagaatcacttggcggcgggtggcgcgctcatgatgtttgtgggcactgttcgacacaaccgctcacagtcatttgcgcaggttgaagcgggtattaagactgcgtactcttcgatggtgaaaacatctcagtggaagaaagaacgtgcacggtacggggtggagcacacctatagtgactatgaggtcacagactcttgggcgaacggttggcacttgcaccgcaacatgctgttgttcttggatcgtccactgtctgacgatgaactcaaggcgtttgaggattccatgttttcccgctggtctgctggtgtggttaaggccggtatggacgcgccactgcgtgagcacggggtcaaacttgatcaggtgtctacctggggtggagacgctgcgaaaatggcaacctacctcgctaagggcatgtctcaggaactgactggctccgctactaaaaccgcgtctaaggggtcgtacacgccgtttcagatgttggatatgttggccgatcaaagcgacgccggcgaggatatggacgctgttttggtggctcggtggcgtgagtatgaggttggttctaaaaacctgcgttcgtcctggtcacgtggggctaagcgtgctttgggcattgattacatagacgctgatgtacgtcgtgaaatggaagaagaactgtacaagctcgccggtctggaagcaccggaacgggtcgaatcaacccgcgttgctgttgctttggtgaagcccgatgattggaaactgattcagtctgatttcgcggttaggcagtacgttctcgattgcgtggataaggctaaggacgtggccgctgcgcaacgtgtcgctaatgaggtgctggcaagtctgggtgtggattccaccccgtgcatgatcgttatggatgatgtggacttggacgcggttctgcctactcatggggacgctactaagcgtgatctgaatgcggcggtgttcgcgggtaatgagcagactattcttcgcacccactaaaagcggcataaaccccgttcgatattttgtgcgatgaatttatggtcaatgtcgcgggggcaaactatgatgggtcttgttgttggcgtcccggaaaacgattccgaagcccaacctttcatagaaggcggcggtggaatttttctccacataagctggcaatgttgcgacgcaacaggtacagtgtaattcatgagaccacgcgtggatccggcttactaaaagccagataacagtatgcgtatttgcgcgctgatttttgcggtataagaatatatactgatatgtatacccgaagtatgtcaaaaagaggtatgctatgaagcagcgtattacagtgacagttgacagcgacagctatcagttgctcaaggcatatatgatgtcaatatctccggtctggtaagcacaaccatgcagaatgaagcccgtcgtctgcgtgccgaacgctggaaagcggaaaatcaggaagggatggctgaggtcgcccggtttattgaaatgaacggctcttttgctgacgagaacaggggctggtgaaatgcagtttaaggtttacacctataaaagagagagccgttatcgtctgtttgtggatgtacagagtgatattattgacacgcccgggcgacggatggtgatccccctggccagtgcacgtctgctgtcagataaagtctcccgtgaactttacccggtggtgcatatcggggatgaaagctggcgcatgatgaccaccgatatggccagtgtgccggtatccgttatcggggaagaagtggctgatctcagccaccgcgaaaatgacatcaaaaacgccattaacctgatgttctggggaatataaggtctcagttttagagctagaaatagcaagttaaaataaggctagtccgttatcaacttgaaaaagtggcaccgagtcggtgctttttttccaggcatcaaataaaacgaaaggctcagtcgaaagactgggcctttcgttttatctgttgtttgtcggtgaacgctctcctgagtaggacaaatccgccgggagcggatttgaacgttgcgaagcaacggcccggagggtggcgggcaggacgcccgccataaactgccaggcatcaaattaagcagaaggccatcctgacggatggcctttttgcgtttctacaaactctttttgtttatttttctaaatacattcaaatatgtatccgctcatgaattaattccgctagatgacgtgcggcttcgaaaatctcgtgatggcaggttgggcgtcgcttggtcggtcatttcgaagggcaccaataactgccttaaaaaaattacgccccgccctgccactcatcgcagtactgttgtaattcattaagcattctgccgacatggaagccatcacagacggcatgatgaacctgaatcgccagcggcatcagcaccttgtcgccttgcgtataatatttgcccatggtgaaaacgggggcgaagaagttgtccatattggccacgtttaaatcaaaactggtgaaactcacccagggattggctgagacgaaaaacatattctcaataaaccctttagggaaataggccaggttttcaccgtaacacgccacatcttgcgaatatatgtgtagaaactgccggaaatcgtcgtggtattcactccagagcgatgaaaacgtttcagtttgctcatggaaaacggtgtaacaagggtgaacactatcccatatcaccagctcaccgtctttcattgccatacggaactccggatgagcattcatcaggcgggcaagaatgtgaataaaggccggataaaacttgtgcttatttttctttacggtctttaaaaaggccgtaatatccagctgaacggtctggttataggtacattgagcaactgactgaaatgcctcaaaatgttctttacgatgccattgggatatatcaacggtggtatatccagtgatttttttctccattttagcttccttagctcctgaaaatctcgtcgaagctcggcggatttgtcctactcaagctgatccgacaaaatccacacattatcccaggtgtccggatcggtcaaatacgctgccagctcatagaccgtatccaaagcatccggggctgatccccggcgccagggtggtttttcttttcaccagtgagacgggcaacagctgattgcccttcaccgcctggccctgagagagttgcagcaagcggtccacgtggtttgccccagcaggcgaaaatcctgtttgatggtggttaacggcgggatataacatgagctgtcttcggtatcgtcgtatcccactaccgagatatccgcaccaacgcgcagcccggactcggtaatggcgcgcattgcgcccagcgccatctgatcgttggcaaccagcatcgcagtgggaacgatgccctcattcagcatttgcatggtttgttgaaaaccggacatggcactccagtcgccttcccgttccgctatcggctgaatttgattgcgagtgagatatttatgccagccagccagacgcagacgcgccgagacagaacttaatgggcccgctaacagcgcgatttgctggtgacccaatgcgaccagatgctccacgcccagtcgcgtaccgtcttcatgggagaaaataatactgttgatgggtgtctggtcagagacatcaagaaataacgccggaacattagtgcaggcagcttccacagcaatggcatcctggtcatccagcggatagttaatgatcagcccactgacgcgttgcgcgagaagattgtgcaccgccgctttacaggcttcgacgccgcttcgttctaccatcgacaccaccacgctggcacccagttgatcggcgcgagatttaatcgccgcgacaatttgcgacggcgcgtgcagggccagactggaggtggcaacgccaatcagcaacgactgtttgcccgccagttgttgtgccacgcggttgggaatgtaattcagctccgccatcgccgcttccactttttcccgcgttttcgcagaaacgtggctggcctggttcaccacgcgggaaacggtctgataagagacaccggcatactctgcgacatcgtataacgttactggtttcacattcaccaccctgaattgactctcttccgggcgctatcatgccataccgcgaaaggttttgcaccattcgatggtgtcaacgtaaatgccgcttcgccttcgcgcgcgaattgcaagctgatccgggcttatcgactgcacggtgcaccaatgcttctggcgtcaggcagccatcggaagctgtggtatggctgtgcaggtcgtaaatcactgcataattcgtgtcgctcaaggcgcactcccgttctggataatgttttttgcgccgacatcataacggttctggcaaatattctgaaatgagctgttgacaattaatcatcggctcgtataatgtgtggaattgtgagcgctcacaatttcacacaggaaacagaatt

SEQ ID NO: 5 - DNA, 807 bp, Artificial Sequence
atgttgtcgtacgagagtatcgacctgtatcgcgaggacgggttcctgttcgcggacccccttaccgaaaaggagacagaccttctacgcgaacaggccgatcgtgagtttctgcgggattctcccggccggatgttggagaaggacggtttcacggtgcgcggggtgcacgggtcgcacgtggtgaacagcacgttcgcccggctggtacggcacccaaagatcgtcacaccggccacgcagctactgggtggccccgtatatgtgcaccagttcaagatcaatgcaaagaaggcgctgaccggcgatgtgtggccctggcaccaggactacatcttctggaaccggggtgacggaatgcgtcgccccgacgtggtgaacgtcgccgtcctgctggatgaggcgaccgatctgaacggtccactgctcgtcctgcccggctcacacaagtgcggctctctggaagtggcgaggcggacgaccgtctgtggcgacggggcgtggcggtccgacatctccgcagatctggactacgccatcgacgcgccgctgctgtccaagctcaccgagactacaaaagtgaccgccatcaaagggccgcccggctcgatcctcctcttcgatcccctgctcgtacacgcctcgggcgtgaacatggctccctacgatcggcgcatgatcctcgtcacctacaaccgggtggacaatccactcggagaggtgcccagccctcgaccggacttcctcgccgcccgggacaacacgccggtcaggccgctcgaccccggcgcggaccttctcgcctaa

SEQ ID NO: 6 - DNA, 24 bp, Artificial Sequence
ttcacactgctcgaacttgtacct

SEQ ID NO: 7 - DNA, 24 bp, Artificial Sequence
aaacaggtacaagttcgagcagtg

SEQ ID NO: 8 - DNA, 78 bp, Artificial Sequence
gcgctcacaatttcacacaggaaacagaattaattaagcttaaaggcacccgatatggataagaaatactcaataggc

SEQ ID NO: 9 - DNA, 27 bp, Artificial Sequence
tcagtcacctcctagctgactcaaatc

SEQ ID NO: 10 - DNA, 42 bp, Artificial Sequence
gtcagctaggaggtgactgaagcttggctgttttggcggatg

SEQ ID NO: 11 - DNA, 30 bp, Artificial Sequence
ctgtgtgaaattgtgagcgctcacaattcc

SEQ ID NO: 12 - DNA, 21 bp, Artificial Sequence
tcgaagggcaccaataactgc

SEQ ID NO: 13 - DNA, 24 bp, Artificial Sequence
cttttactttcaccagcgtttctg

SEQ ID NO: 14 - DNA, 24 bp, Artificial Sequence
aacgctggtgaaagtaaaagatgc

SEQ ID NO: 15 - DNA, 45 bp, Artificial Sequence
gaatggaacggatcaaacggtgaattacactgtacctgttgcgtc

SEQ ID NO: 16 - DNA, 43 bp, Artificial Sequence
ccgtttgatccgttccattcgttttagagctagaaatagcaag

SEQ ID NO: 17 - DNA, 23 bp, Artificial Sequence
caacctgccatcacgagattttc

SEQ ID NO: 18 - DNA, 40 bp, Artificial Sequence
aatctcgtgatggcaggttgacgggagcctaagtgaaatg

SEQ ID NO: 19 - DNA, 41 bp, Artificial Sequence
ccttggtaaatgcacggtatgggtcagtgagatcaatcggg

SEQ ID NO: 20 - DNA, 22 bp, Artificial Sequence
ccataccgtgcatttaccaagg

SEQ ID NO: 21 - DNA, 40 bp, Artificial Sequence
cagttattggtgcccttcgactttgtggtcttctttgcgg

SEQ ID NO: 22 - DNA, 39 bp, Artificial Sequence
acaggccaaaggagttgagaatgttgagttttgcgaccc

SEQ ID NO: 23 - DNA, 40 bp, Artificial Sequence
ccaagcttgcatgcctgcagttaccttttattaccgaatc